European Patent Application EP 4 736 664 A1, published May 6, 2026. Title: COMPOSITION FOR SUBSTITUTING EGG WHITE. Applicant: 味の素株式会社. Application WO. The sequence listing filed with the application follows.

SEQUENCE LISTING (19 sequences)

SEQ ID NO: 1 - DNA, 1173 bp, Arabidopsis thaliana
  source 1..1173: mol_type = genomic DNA
atggatgtgcgtgaaagcattagtctgcagaatcaggtgtctatgaatctcgcgaaacacgtcattaccacggtaagccagaattccaacgtcattttcagtcccgcttcgattaacgtcgtgctgtctattatcgcagcgggcagtgcaggagccaccaaagatcagattctgagttttctgaaatttagttctactgaccagttgaacagcttttcctcggaaatcgtgtcagccgttcttgctgatggtagcgccaatggtggccctaaactgtcggtagcaaatggggcgtggattgacaaatctctgtccttcaaaccgtcatttaagcagcttctggaagattcctacaaggcggcatctaaccaagccgactttcaatcaaaagccgtcgaagttattgctgaggttaacagctgggcagagaaagaaacgaatggcctgattacggaggtgcttcccgaaggaagcgctgatagcatgaccaagctgatcttcgctaacgcgctgtactttaaagggacctggaacgagaaatttgatgagagcctcacccaagaaggcgaatttcacttactggacggcaacaaagttactgcgccttttatgacgtcgaagaagaaacagtatgtatccgcctatgacggctttaaagtgttagggttgccgtatctgcagggtcaggacaaacggcaattctcgatgtacttctatctcccggatgcgaataacggcttgtcggatttactggataaaatcgtttccacaccaggcttcctggacaatcatatcccacgtcgccaggtgaaggttcgcgaattcaaaattccgaaattcaaattcagctttggcttcgatgcgagcaatgtcttgaaaggtctgggcttaacgagtccgttttcaggcgaagaaggtttgacagaaatggttgaatctccagaaatggggaagaatctgtgtgtgagcaacatctttcacaaagcctgcattgaagtgaacgaggaaggtactgaggcggcagccgcatcagcgggtgtgatcaaattacgcggacttctcatggaagaagatgaaatcgactttgtcgcggatcatccgttcctgctggttgtcaccgagaacattaccggtgtggtactgtttatcggtcaagtggtagatccgctgcat

SEQ ID NO: 2 - protein, 391 aa, Arabidopsis thaliana
MDVRESISLQNQVSMNLAKHVITTVSQNSNVIFSPASINVVLSIIAAGSAGATKDQILSFLKFSSTDQLNSFSSEIVSAVLADGSANGGPKLSVANGAWIDKSLSFKPSFKQLLEDSYKAASNQADFQSKAVEVIAEVNSWAEKETNGLITEVLPEGSADSMTKLIFANALYFKGTWNEKFDESLTQEGEFHLLDGNKVTAPFMTSKKKQYVSAYDGFKVLGLPYLQGQDKRQFSMYFYLPDANNGLSDLLDKIVSTPGFLDNHIPRRQVKVREFKIPKFKFSFGFDASNVLKGLGLTSPFSGEEGLTEMVESPEMGKNLCVSNIFHKACIEVNEEGTEAAAASAGVIKLRGLLMEEDEIDFVADHPFLLVVTENITGVVLFIGQVVDPLH

SEQ ID NO: 3 - DNA, 1176 bp, Brassica napus
  source 1..1176: mol_type = genomic DNA
atggacgtacgggagagcatttcgctgcagaatcatgtgtcgttgtcactggcgaaaaacgtgatttcgacggtaagcaaaaactcgaatgtcattttctcaccggcatcgattaacgtcgttctgggcattattgcggcaggtagtgcaggtgcaaccaaagaccagattctgtcctttctgaactttccctcaatcgaccatttgaacaccttttcatccgatatcgtaagtgcggttctggccgatggtagtgccaatggtggcccaaaactgtcagccgcaaatggtgtttggattgataagagcctctcctttaaaccgagcttcaagcagctcttggatgggagttacaaagctgcgagcaatctcgcggatttccagacgaaagcggtcgaagtcatcgctgaagtgaattcttgggccgaaaaagaaaccaatggtctgataaccgaagtgctgccagaaggttctgcagactccatgactcgcctgatttttgcgaatgcgctgtactttaaggggacttggaacgagaaattcgacgagtcgctgaccaaagatggcgattttcaccttctggacgggagttccaaagttacagccccattcatgacgagcaagaaaaagcagtatgttagcgcttatgaaggctttaaggtgttagggcttccgtatcttcaaggcgaagataagcgccaattctctatgtacctgtatttgcctgatgccaataacggcttgagcgatttactggacaaaatcgtatccacccctggttttctggattctcacataccgcgtcgtcaagtcaaagttggcgagttcaaaatccccaaattcaaattcagctttggctttgaagcgagtgatgtgcttaaaggcttagggctgacatctccgtttagcggcgaagatggtctaaccgaaatggtggaaagcccggaaatgggcaaaaacctgaaagtgagctcgatctttcacaaagcctgcatcgaagtgaacgaggaaggaactgaagctgcggcagcttctgccggtgtgatcaaactgcgcggattagcgatggaggaagagattatcgactttgttgccgaccatccgttcctgttagtggtcatggagaacattacgggcgttattctcttcatcggacaggtaattgatccgctacat

SEQ ID NO: 4 - protein, 392 aa, Brassica napus
MDVRESISLQNHVSLSLAKNVISTVSKNSNVIFSPASINVVLGIIAAGSAGATKDQILSFLNFPSIDHLNTFSSDIVSAVLADGSANGGPKLSAANGVWIDKSLSFKPSFKQLLDGSYKAASNLADFQTKAVEVIAEVNSWAEKETNGLITEVLPEGSADSMTRLIFANALYFKGTWNEKFDESLTKDGDFHLLDGSSKVTAPFMTSKKKQYVSAYEGFKVLGLPYLQGEDKRQFSMYLYLPDANNGLSDLLDKIVSTPGFLDSHIPRRQVKVGEFKIPKFKFSFGFEASDVLKGLGLTSPFSGEDGLTEMVESPEMGKNLKVSSIFHKACIEVNEEGTEAAAASAGVIKLRGLAMEEEIIDFVADHPFLLVVMENITGVILFIGQVIDPLH

SEQ ID NO: 5 - DNA, 1170 bp, Theobroma cacao
  source 1..1170: mol_type = genomic DNA
atggatctgcgtgagagcattcgccgtcagaccgatgtgacgcttagtttgacgaaacatgtgttacagactgaggcaaaagattccaatctggccttctcaccattgtccattcacgttgtactctcaatgattgcggcgggctctaccgggcctaccctggatcagctgctctcgttcctgaaaagcgcaagcaacgatcacctgggtagctttagctcggaactggtgtcagtggtgtttgccgatggctctccagccggaggcccgcgcttgtcatttgccaatggggtttggatcgataagagtctgccgctgaaaccgagctttaaacaggtggtcgacaacgtgtataaagcagccagtaatcaggtggactttcagaccaaagcggtgcaagtagcgggtgaagttaacctttgggctgagaaagaaacatcgggtctgattaagcagttactccctcctggctccgttgatggctctactcggctgatcttcgccaatgccttgtactttaaaggcgcatggaacgaaacctttgatgcttccaaaacgaaagaaaacgacttctacttggtcaatggcagtagtgtgaaagcgccatttatgacctcgcagaagaagcaagcggtaggtgcgtatgacggctttaaagtcctgggtttaccctataagcaaggcggtgacaaacgccgcttctcaatgtacttcttccttccggatgcgaaagatgggctgccagcattagtggagaaagtctcgtctgaatccgggttcctggagcgccatctgccgtatgaaccggtgaaagttggggagtttcgcattccgcggttcaaaatcagctttggttttgaagccagcgaagtgttgaaacgtctgggactggtcctgccgttttctggtgaaggcggcttaacggaaatggtagatagcccgttaggtcaaagcctgtatgtttccaacatctttcacaaatcgttcatcgaagtcaacgaggaaggcacagaagcggctgctgcaagtgctggtgtgattcgtctgcgcggtgtcctggttgaagaaaagattgactttgtagcggatcatccgttcctctttctgattcgtgaggacgttaccggcgtcgtactcttcatcggacatgttctgaatccccttgaaagc

SEQ ID NO: 6 - protein, 390 aa, Theobroma cacao
MDLRESIRRQTDVTLSLTKHVLQTEAKDSNLAFSPLSIHVVLSMIAAGSTGPTLDQLLSFLKSASNDHLGSFSSELVSVVFADGSPAGGPRLSFANGVWIDKSLPLKPSFKQVVDNVYKAASNQVDFQTKAVQVAGEVNLWAEKETSGLIKQLLPPGSVDGSTRLIFANALYFKGAWNETFDASKTKENDFYLVNGSSVKAPFMTSQKKQAVGAYDGFKVLGLPYKQGGDKRRFSMYFFLPDAKDGLPALVEKVSSESGFLERHLPYEPVKVGEFRIPRFKISFGFEASEVLKRLGLVLPFSGEGGLTEMVDSPLGQSLYVSNIFHKSFIEVNEEGTEAAAASAGVIRLRGVLVEEKIDFVADHPFLFLIREDVTGVVLFIGHVLNPLES

SEQ ID NO: 7 - DNA, 1173 bp, Ricinus communis
  source 1..1173: mol_type = genomic DNA
atggatttacgcgagtcaatcaagaaccagattgacgtggctctgacgctgagtaaacatgttctcctgggtgaagccaaatcgtccaactcggtgttttctccgctgagtattcaggttgtactcggcattattgctgccggctcgaaaggcgccactttggaccagctgttatcgtttctgaaatctaaatcgaacgatcagctgagcagctttagttccgaacttgtcgctgtggcgtttgcggatggtagtgcagccggtggtcctcgcctctccttcgctaatggggtttgggtagataaggcgttaagcctgaaacactctttcaagcaagtcgttgataacgtgtataaggcggcaagtaataacgtggatttccaaaccaaagcggtggaagtagccaatgaggtgaatgcatgggcagagaaagaaactgatggcttgatcaaagaagtcctgcctagcggctctgtggacaattctacccgtttagtctttgccaatgccctgtactttaaaggcgcgtggaccgagaaattcgatgcgagcatcaccaaagaccatgacttctatctgctgaacggcagctccgtacatgcgccgtttatgaccagcaagaagaaacagttcattcgcgcttttgaaggcttcaaagtcttgggcctgccgtattaccagggacaggataaacgccagtttagcatgtacttcttcctgcccgatgccaaagacgggctgccggcactggtggagaaagttggaagtgaatcaggttttcttgatcaccatttaccacgtcaacaagtggaagtcggtgattttcggattccacgctttcgtattagctttgggttcgaagcaagcgaagcgctgaaaggcttgggcttagtgcttccctttagcggtgagggtgaccttacggaaatggtggatagctccgttgggcagaaactgtatgtctcatccatctttcacaaatctttcatcgaagttaacgaggaaggcacagaagcggcggcagcttcagccggtgtgatcaaactgcgttcgctggcgttttcggacaagattgacttcgttgccgatcacccgtttctgttcctgattcgcgaaaacatgacgggtttggtactctttatcggacatgttctggaaccgtcacaagcgaat

SEQ ID NO: 8 - protein, 391 aa, Ricinus communis
MDLRESIKNQIDVALTLSKHVLLGEAKSSNSVFSPLSIQVVLGIIAAGSKGATLDQLLSFLKSKSNDQLSSFSSELVAVAFADGSAAGGPRLSFANGVWVDKALSLKHSFKQVVDNVYKAASNNVDFQTKAVEVANEVNAWAEKETDGLIKEVLPSGSVDNSTRLVFANALYFKGAWTEKFDASITKDHDFYLLNGSSVHAPFMTSKKKQFIRAFEGFKVLGLPYYQGQDKRQFSMYFFLPDAKDGLPALVEKVGSESGFLDHHLPRQQVEVGDFRIPRFRISFGFEASEALKGLGLVLPFSGEGDLTEMVDSSVGQKLYVSSIFHKSFIEVNEEGTEAAAASAGVIKLRSLAFSDKIDFVADHPFLFLIRENMTGLVLFIGHVLEPSQAN

SEQ ID NO: 9 - DNA, 1125 bp, Brassica rapa subsp. pekinensis
  source 1..1125: mol_type = genomic DNA
atggacttacaggaatccgtgcggaaacagaacgggattttatggcgcgtctacaaacacgtcattaacaccactgcgggtaagacgtcgaacttagtcatcagtccagcactcattagcgtaatcctgtcattcattgcggcctataaatctcctggtgcaacggaagaacagatcctgtctctgctcaaagcctcaagtaccgatgaattgaatgcagtgagcagtcagatcgttaccactgtgctcgcagatagtaccacgtcaggtggcccgatgatcagcacagctaacgggttttggattgagaaaagcctgtgctgtgtggaacagtctttcaagaatcttctggaaactagctacaaagccgcgtttaaacaggtggattttcgcaccaaagcggacgaagtaagcgaagaagtgaacacgtgggtggagaaacagaccaatggactgattaccggcttactcccgggtccagcctataaaggcggtcaagcggttcgtccgccaggttcggagccggtgtctcccgtatgggacgaggaatttgatccgagccttacgaaagactccgactttcatttgctggacggcacaaaagttccagtgccgtttatgtccggcgatttcttttcgtatcatctggatgtgtatccgggctttaaagtcctgaatctgccctatcgcgaaggacgtcgtgatggtcgctctttctcgatgcaaatctaccttcctgatgaaaaggaaggtttaccggcgatgcttgagatgctggccagtaccccggaagatgaagatgaggatattccctcatatcgcgcggatattggggaactgaagatccctaaattcaaatttggctttcactttgaggccacagaagcgctgaaatcgttgggtctgagcctgcctctggaaaccattttccacaaatcctgcattgaagttgacgaagtaggcagcaaagctgctgctgcagccgcggttgttggggagggctgctgtggaccggcagaaaagaagtacgactttgtcgcggatcatccgttcctgttcctggtgaaagagcatggctccggcgttgtcctgttcttgggtcaagttctggatccgagcatgcat

SEQ ID NO: 10 - protein, 375 aa, Brassica rapa subsp. pekinensis
MDLQESVRKQNGILWRVYKHVINTTAGKTSNLVISPALISVILSFIAAYKSPGATEEQILSLLKASSTDELNAVSSQIVTTVLADSTTSGGPMISTANGFWIEKSLCCVEQSFKNLLETSYKAAFKQVDFRTKADEVSEEVNTWVEKQTNGLITGLLPGPAYKGGQAVRPPGSEPVSPVWDEEFDPSLTKDSDFHLLDGTKVPVPFMSGDFFSYHLDVYPGFKVLNLPYREGRRDGRSFSMQIYLPDEKEGLPAMLEMLASTPEDEDEDIPSYRADIGELKIPKFKFGFHFEATEALKSLGLSLPLETIFHKSCIEVDEVGSKAAAAAAVVGEGCCGPAEKKYDFVADHPFLFLVKEHGSGVVLFLGQVLDPSMH

SEQ ID NO: 11 - DNA, 1122 bp, Raphanus sativus
  source 1..1122: mol_type = genomic DNA
atggatgcgaaagagagcatgaagaagcagaacgagttggccatgttccttgcccgtcatgtgttttcttcagaagcaaaacacagcaatatcgtcttttctcctgcgagtatctatagcgcgttgaccctggttgcatccgcgcccagcgaacccagtgttgcagacgaaatcctttgctttctcaaatcctcttcaaccgacgaattgaatgcagtgttcacggagctggtgagcttggtatatacgggtggtaacgcgtcgggtggaccggaaatttcatcggttaatggcgtttggattgagaaaaccatctctctggatccgaaactcaaagacctgttagagaacttcttcaaagcggcttttaacctggtcgactttgtatctaaatccgaagaagtgcgcattgaagttaactcatgggtacaggaacgcacgaatgatctcatcaaggatctgctgccgcctgggagtgttacgaacaagactgaacggatttatgcgaatgccctgtacttcaaaggcacctggcaaacaccgttcgacgactacgatactcgtaaacgcaaattttacctgttaaacggatcgaccgtcagtgtcccgtttatgacctcgggtgaggatcagtatattgcggcgtatgatggattcaaagtcgcacgtttaccgtttcaaggcggtcgtggggacacgaatcgcacttttgccatgtacttctatctgccacgcaagaaagatgggcttgacaatctggtggaacgtattgcgacaactccaggcttcctggatgcccatgttccaggttgcgaggtgaaagtgggcacctttcgcattcctaaattcgaaatctcctttggctttctggtgagcgatgtgttctcgcaactggaactgggcagcaactcgctgtatcacaaagcctttatcaaaattgatgaaagcggcgtagaagctgctgcagctacggctgatgaagcgtgtggctgttacttaggcatggaaccgccgaagtccattgacttcgtcgccaacaaaccgtttctgtttctcattcgcaaagatacaaccggtaccgtgctgtttgccggtcagatctttgatccgagccagagtagc

SEQ ID NO: 12 - protein, 374 aa, Raphanus sativus
MDAKESMKKQNELAMFLARHVFSSEAKHSNIVFSPASIYSALTLVASAPSEPSVADEILCFLKSSSTDELNAVFTELVSLVYTGGNASGGPEISSVNGVWIEKTISLDPKLKDLLENFFKAAFNLVDFVSKSEEVRIEVNSWVQERTNDLIKDLLPPGSVTNKTERIYANALYFKGTWQTPFDDYDTRKRKFYLLNGSTVSVPFMTSGEDQYIAAYDGFKVARLPFQGGRGDTNRTFAMYFYLPRKKDGLDNLVERIATTPGFLDAHVPGCEVKVGTFRIPKFEISFGFLVSDVFSQLELGSNSLYHKAFIKIDESGVEAAAATADEACGCYLGMEPPKSIDFVANKPFLFLIRKDTTGTVLFAGQIFDPSQSS

SEQ ID NO: 13 - DNA, 1230 bp, Helianthus annuus
  source 1..1230: mol_type = genomic DNA
atggcggaagccatggacttcaaacaaagcattcgggaccagacgcatgtatccacgaccctggcagctcatctgctgagtaagaaacacgatagtaacgtagtgttcagcccggtgtcaattcacgccgtacttagcttgttggcccaagggaccactggtcgtacccgcgatcagctgcttgcctttctgaaaaccaatacgacgcataacctgaattcgctgtattcgcaatacgtgtcaagtatcttcggggatagcagctctacagatggtccacgtctgtctagcatctttggggatagttcatcaagcgatggaccacgcctgagcattgcgaatggcgtttgggtggacaaaacgttgtccctcaaaccgtcgtttaaacaggtggtagatgatgtttataaggccgtgtgcaaacaggtcgactttcagaccaaagcggcggaggtagtggatgaagtgaacttgtgggcggaacgccagactaatggtctgattaaggaattattacacgcagatgaagtctccagcttaacgcgcttaatcttcgcgaatgcgctgtacttcaaaggcacttggcgtgatccgtttgaccgtgaggcgaccattgagtcggactttcaccttttgggaggtaacaaggtgcaagttccctttatgaccgataacgagttcaaatttgtatgcgaatacgatgactttaaggtcctgggccttccgtatctgcgtggtcaagaacgccgcgagttcaccatgtacttctttctgccgaatgctaaagacggcctgcagagcttagttcagaaaatcgggtctacctctgactttctggattcgcatattcggggccaacaggtggaagttggccgctttctcctgccgaaattcaaaatcgaatttcgctttaaagtctgcgacatgctgatggaactgggcttagtcctgccctttacaggtgaagatggactcaccgaaatggcggattcgagtgcaggcgaacgtctgcatgtttcatccattcaccagaaaagtttcatggaagtgaacgaagagggcactgaagcagctgcagtgacctatgagcagtgttatggttgtgcttccgacgaagaagaacctcgtcgcgtcgattttgttgccgatcatccgttcctgttcgttattcgcgaggatgttacaggtgttgtgctctttgtgggtcaggtcatcaacccttctgtcggc

SEQ ID NO: 14 - protein, 410 aa, Helianthus annuus
MAEAMDFKQSIRDQTHVSTTLAAHLLSKKHDSNVVFSPVSIHAVLSLLAQGTTGRTRDQLLAFLKTNTTHNLNSLYSQYVSSIFGDSSSTDGPRLSSIFGDSSSSDGPRLSIANGVWVDKTLSLKPSFKQVVDDVYKAVCKQVDFQTKAAEVVDEVNLWAERQTNGLIKELLHADEVSSLTRLIFANALYFKGTWRDPFDREATIESDFHLLGGNKVQVPFMTDNEFKFVCEYDDFKVLGLPYLRGQERREFTMYFFLPNAKDGLQSLVQKIGSTSDFLDSHIRGQQVEVGRFLLPKFKIEFRFKVCDMLMELGLVLPFTGEDGLTEMADSSAGERLHVSSIHQKSFMEVNEEGTEAAAVTYEQCYGCASDEEEPRRVDFVADHPFLFVIREDVTGVVLFVGQVINPSVG

SEQ ID NO: 15 - DNA, 1116 bp, Camellia sinensis var. sinensis
  source 1..1116: mol_type = genomic DNA
atggaaaaccaagtcctgttaaaacagatcgacaaagggtctaacttcgtactctccccactttcgttccacttcatgttgagcttgattgctagtggttcaaccggtcgtactctgaaacaacttctgtcgtatctggggagtaagtccattggtgacttgaacttcatgagcagccagtttatcccgcttacctcgatgatgtccaatgtcaaaggaggtaaaaacaagaataaccagatcagttctccgagcatatcctttgcgaatggcttatggattgatcgtcgttttagcctctcaccgtcttacgaacgcattctgaaagcgagctatgacgcaaaagccaatgaagtcgattttgccaacaagaatctgatggaaagtggctatggcttcaatgaactatgctttaactttccgcaaaatctgcagcagaagacgcagaatcagtgcttcgataacaacggcttactgagcaagaacaacaaccatcagtctatgcccttctcgcagtcaattgctgttcagatcgaaaaacagcgtcaagagattgatcgcgtaatctcactgcagaatgagcgattacggttgacgttacaggaacagcgtaaacaacagatcgcgcttattctgcgcaaatacgaagtgaagaccctggttttgctgaaccaaaaagacgaggaaatagccaaagcgatgaatcgggccatggaactggaggactttctgcgccgcatggaaatcgagaatcagacgtggcaaagagtggcaaaagaaaacgaggcaatggtagtgtcgctcaataacaccatcaaacaactgcgcgaaaacgcgtgtctggttgatggcattgaagatgctgagtcgtgttgtgatgtgatgatttatcgtggcgataatgaaacaggcgaaaaccgtggatacgagaaaaaccagcaggagaatgaagaacaaggtactcgcaaaatggtttgcaaatcctgcaattctcgcaacagttgcgtgatctttctgccttgtcgtcatctgtgcagctgtaaagcctgccaagcgtttctggatagctgcccagtgtgtggtatggccaaaaaagcgagcattgaagcactcatt

SEQ ID NO: 16 - protein, 372 aa, Camellia sinensis var. sinensis
MENQVLLKQIDKGSNFVLSPLSFHFMLSLIASGSTGRTLKQLLSYLGSKSIGDLNFMSSQFIPLTSMMSNVKGGKNKNNQISSPSISFANGLWIDRRFSLSPSYERILKASYDAKANEVDFANKNLMESGYGFNELCFNFPQNLQQKTQNQCFDNNGLLSKNNNHQSMPFSQSIAVQIEKQRQEIDRVISLQNERLRLTLQEQRKQQIALILRKYEVKTLVLLNQKDEEIAKAMNRAMELEDFLRRMEIENQTWQRVAKENEAMVVSLNNTIKQLRENACLVDGIEDAESCCDVMIYRGDNETGENRGYEKNQQENEEQGTRKMVCKSCNSRNSCVIFLPCRHLCSCKACQAFLDSCPVCGMAKKASIEALI

SEQ ID NO: 17 - DNA, 1254 bp, Daucus carota subsp. sativus
  source 1..1254: mol_type = genomic DNA
atgcgccccactgggactaaaccgattacaccgaaaatcgaaatggaccagattatctccaaccagacagacgtcgccatgacgttaaccaaacacattctgggcgataacaatccgtgcaatgtggttctttctcccctgagcctgcagctggtacttggtctggttgcagctgggtcggaatcagagtcattgaagcaactgctctcgttcttaaaagcggaatctactgaagagttgaactcgctggctagtcatctggcgaatcacgttttcacaggcggttcaccgccgggagaactgactctgagcttagcgaacggtgtttggattgacaaatccctttcttttcagcccttctttagcaaggtggtcgatgatgtctataaagcgggaagcgatgtggtggatttcaagaacaaagccagtgaagctgccgagaaggtcaatttgtggatcgaaaagaaaacgtatggcctgatcaaagacaccattagccctgacctgttcgatgatgaaacccggatcgtgtttgcgaacgccatctatttcaaaggcttttgggcaaacaaatttgatatgctgtcgacccgtaacgacgatttctacctgttagatgatagcagtgttcatgtcccgtttatgaccagtaccacgaaatactattgcatttcggcgtttgatgggttcaaagtgctggagttgccgtataaacgcgaaaccgatatgcgggacatttctatgtacttcttcctgccagatgcgaaagatggcctgagcaccttggtagacaaactggcaagtgagtcgggttttctggaacgccacattccgtccgagatggaacgtgtcggacaactgcgcattccgaagtttaaaatcagctttgaatttgaagcgtctaaagccctcaaagaattaggtgtgtgtgcaccattcattcgtgggcgtcgtgatttcgatcgtatggttaattccgtgtatgacgagttactgtatgtgtccggtgtatttcaggagagctacattgaagttaacgaaagtggtacggaagcatgcgcgtacagccgcattcctatgtgtggcggtggcccactccctgtgaccaaaatcgactttatcgctgatcatccgtttctgtttcttattcgcgaaaacaaaacgggcgttgtgctctttatcggccaagtactgaatccggaagcctcatggccacgcttttcaattgactacaatacgatcttcggcaatcgc

SEQ ID NO: 18 - protein, 418 aa, Daucus carota subsp. sativus
MRPTGTKPITPKIEMDQIISNQTDVAMTLTKHILGDNNPCNVVLSPLSLQLVLGLVAAGSESESLKQLLSFLKAESTEELNSLASHLANHVFTGGSPPGELTLSLANGVWIDKSLSFQPFFSKVVDDVYKAGSDVVDFKNKASEAAEKVNLWIEKKTYGLIKDTISPDLFDDETRIVFANAIYFKGFWANKFDMLSTRNDDFYLLDDSSVHVPFMTSTTKYYCISAFDGFKVLELPYKRETDMRDISMYFFLPDAKDGLSTLVDKLASESGFLERHIPSEMERVGQLRIPKFKISFEFEASKALKELGVCAPFIRGRRDFDRMVNSVYDELLYVSGVFQESYIEVNESGTEACAYSRIPMCGGGPLPVTKIDFIADHPFLFLIRENKTGVVLFIGQVLNPEASWPRFSIDYNTIFGNR

SEQ ID NO: 19 - DNA, 5442 bp, synthetic construct
  source 1..5442: mol_type = other DNA
  misc_feature 1..5442: note = pET21b(+)
tggcgaatgggacgcgccctgtagcggcgcattaagcgcggcgggtgtggtggttacgcgcagcgtgaccgctacacttgccagcgccctagcgcccgctcctttcgctttcttcccttcctttctcgccacgttcgccggctttccccgtcaagctctaaatcgggggctccctttagggttccgatttagtgctttacggcacctcgaccccaaaaaacttgattagggtgatggttcacgtagtgggccatcgccctgatagacggtttttcgccctttgacgttggagtccacgttctttaatagtggactcttgttccaaactggaacaacactcaaccctatctcggtctattcttttgatttataagggattttgccgatttcggcctattggttaaaaaatgagctgatttaacaaaaatttaacgcgaattttaacaaaatattaacgtttacaatttcaggtggcacttttcggggaaatgtgcgcggaacccctatttgtttatttttctaaatacattcaaatatgtatccgctcatgagacaataaccctgataaatgcttcaataatattgaaaaaggaagagtatgagtattcaacatttccgtgtcgcccttattcccttttttgcggcattttgccttcctgtttttgctcacccagaaacgctggtgaaagtaaaagatgctgaagatcagttgggtgcacgagtgggttacatcgaactggatctcaacagcggtaagatccttgagagttttcgccccgaagaacgttttccaatgatgagcacttttaaagttctgctatgtggcgcggtattatcccgtattgacgccgggcaagagcaactcggtcgccgcatacactattctcagaatgacttggttgagtactcaccagtcacagaaaagcatcttacggatggcatgacagtaagagaattatgcagtgctgccataaccatgagtgataacactgcggccaacttacttctgacaacgatcggaggaccgaaggagctaaccgcttttttgcacaacatgggggatcatgtaactcgccttgatcgttgggaaccggagctgaatgaagccataccaaacgacgagcgtgacaccacgatgcctgcagcaatggcaacaacgttgcgcaaactattaactggcgaactacttactctagcttcccggcaacaattaatagactggatggaggcggataaagttgcaggaccacttctgcgctcggcccttccggctggctggtttattgctgataaatctggagccggtgagcgtgggtctcgcggtatcattgcagcactggggccagatggtaagccctcccgtatcgtagttatctacacgacggggagtcaggcaactatggatgaacgaaatagacagatcgctgagataggtgcctcactgattaagcattggtaactgtcagaccaagtttactcatatatactttagattgatttaaaacttcatttttaatttaaaaggatctaggtgaagatcctttttgataatctcatgaccaaaatcccttaacgtgagttttcgttccactgagcgtcagaccccgtagaaaagatcaaaggatcttcttgagatcctttttttctgcgcgtaatctgctgcttgcaaacaaaaaaaccaccgctaccagcggtggtttgtttgccggatcaagagctaccaactctttttccgaaggtaactggcttcagcagagcgcagataccaaatactgtccttctagtgtagccgtagttaggccaccacttcaagaactctgtagcaccgcctacatacctcgctctgctaatcctgttaccagtggctgctgccagtggcgataagtcgtgtcttaccgggttggactcaagacgatagttaccggataaggcgcagcggtcgggctgaacggggggttcgtgcacacagcccagcttggagcgaacgacctacaccgaactgagatacctacagcgtgagctatgagaaagcgccacgcttcccgaagggagaaaggcggacaggtatccggtaagcggcagggtcggaacaggagagcgcacgagggagcttccagggggaaacgcctggtatctttatagtcctgtcgggtttcgccacctctgacttgagcgtcgatttttgtgatgctcgtcaggggggcggagcctatggaaaaacgccagcaacgcggcctttttacggttcctggccttttgctggccttttgctcacatgttctttcctgcgttatcccctgattctgtggataaccgtattaccgcctttgagtgagctgataccgctcgccgcagccgaacgaccgagcgcagcgagtcagtgagcgaggaagcggaagagcgcctgatgcggtattttctccttacgcatctgtgcggtatttcacaccgcatatatggtgcactctcagtacaatctgctctgatgccgcatagttaagccagtatacactccgctatcgctacgtgactgggtcatggctgcgccccgacacccgccaacacccgctgacgcgccctgacgggcttgtctgctcccggcatccgcttacagacaagctgtgaccgtctccgggagctgcatgtgtcagaggttttcaccgtcatcaccgaaacgcgcgaggcagctgcggtaaagctcatcagcgtggtcgtgaagcgattcacagatgtctgcctgttcatccgcgtccagctcgttgagtttctccagaagcgttaatgtctggcttctgataaagcgggccatgttaagggcggttttttcctgtttggtcactgatgcctccgtgtaagggggatttctgttcatgggggtaatgataccgatgaaacgagagaggatgctcacgatacgggttactgatgatgaacatgcccggttactggaacgttgtgagggtaaacaactggcggtatggatgcggcgggaccagagaaaaatcactcagggtcaatgccagcgcttcgttaatacagatgtaggtgttccacagggtagccagcagcatcctgcgatgcagatccggaacataatggtgcagggcgctgacttccgcgtttccagactttacgaaacacggaaaccgaagaccattcatgttgttgctcaggtcgcagacgttttgcagcagcagtcgcttcacgttcgctcgcgtatcggtgattcattctgctaaccagtaaggcaaccccgccagcctagccgggtcctcaacgacaggagcacgatcatgcgcacccgtggggccgccatgccggcgataatggcctgcttctcgccgaaacgtttggtggcgggaccagtgacgaaggcttgagcgagggcgtgcaagattccgaataccgcaagcgacaggccgatcatcgtcgcgctccagcgaaagcggtcctcgccgaaaatgacccagagcgctgccggcacctgtcctacgagttgcatgataaagaagacagtcataagtgcggcgacgatagtcatgccccgcgcccaccggaaggagctgactgggttgaaggctctcaagggcatcggtcgagatcccggtgcctaatgagtgagctaacttacattaattgcgttgcgctcactgcccgctttccagtcgggaaacctgtcgtgccagctgcattaatgaatcggccaacgcgcggggagaggcggtttgcgtattgggcgccagggtggtttttcttttcaccagtgagacgggcaacagctgattgcccttcaccgcctggccctgagagagttgcagcaagcggtccacgctggtttgccccagcaggcgaaaatcctgtttgatggtggttaacggcgggatataacatgagctgtcttcggtatcgtcgtatcccactaccgagatatccgcaccaacgcgcagcccggactcggtaatggcgcgcattgcgcccagcgccatctgatcgttggcaaccagcatcgcagtgggaacgatgccctcattcagcatttgcatggtttgttgaaaaccggacatggcactccagtcgccttcccgttccgctatcggctgaatttgattgcgagtgagatatttatgccagccagccagacgcagacgcgccgagacagaacttaatgggcccgctaacagcgcgatttgctggtgacccaatgcgaccagatgctccacgcccagtcgcgtaccgtcttcatgggagaaaataatactgttgatgggtgtctggtcagagacatcaagaaataacgccggaacattagtgcaggcagcttccacagcaatggcatcctggtcatccagcggatagttaatgatcagcccactgacgcgttgcgcgagaagattgtgcaccgccgctttacaggcttcgacgccgcttcgttctaccatcgacaccaccacgctggcacccagttgatcggcgcgagatttaatcgccgcgacaatttgcgacggcgcgtgcagggccagactggaggtggcaacgccaatcagcaacgactgtttgcccgccagttgttgtgccacgcggttgggaatgtaattcagctccgccatcgccgcttccactttttcccgcgttttcgcagaaacgtggctggcctggttcaccacgcgggaaacggtctgataagagacaccggcatactctgcgacatcgtataacgttactggtttcacattcaccaccctgaattgactctcttccgggcgctatcatgccataccgcgaaaggttttgcgccattcgatggtgtccgggatctcgacgctctcccttatgcgactcctgcattaggaagcagcccagtagtaggttgaggccgttgagcaccgccgccgcaaggaatggtgcatgcaaggagatggcgcccaacagtcccccggccacggggcctgccaccatacccacgccgaaacaagcgctcatgagcccgaagtggcgagcccgatcttccccatcggtgatgtcggcgatataggcgccagcaaccgcacctgtggcgccggtgatgccggccacgatgcgtccggcgtagaggatcgagatctcgatcccgcgaaattaatacgactcactataggggaattgtgagcggataacaattcccctctagaaataattttgtttaactttaagaaggagatatacatatggctagcatgactggtggacagcaaatgggtcgggatccgaattcgagctccgtcgacaagcttgcggccgcactcgagcaccaccaccaccaccactgagatccggctgctaacaaagcccgaaaggaagctgagttggctgctgccaccgctgagcaataactagcataaccccttggggcctctaaacgggtcttgaggggttttttgctgaaaggaggaactatatccggat